European Patent Application EP 4 122 493 A1, published January 25, 2023. Title: METHOD FOR TREATING CHOLESTEROL-RELATED DISEASES. Applicant: JIANGSU HENGRUI PHARMACEUTICALS CO., LTD. The sequence listing filed with the application follows.

SEQUENCE LISTING (10 sequences)

SEQ ID NO: 1 - protein, 5 aa, Artificial Sequence
  HCDR1
DYWMH

SEQ ID NO: 2 - protein, 17 aa, Artificial Sequence
  HCDR2
YINPSSGFTKYHQNFKD

SEQ ID NO: 3 - protein, 12 aa, Artificial Sequence
  HCDR3
QYDYDEDWYFDV

SEQ ID NO: 4 - protein, 17 aa, Artificial Sequence
  LCDR1
KSSQSLLNSRTRKNFLA

SEQ ID NO: 5 - protein, 7 aa, Artificial Sequence
  LCDR2
WASTRES

SEQ ID NO: 6 - protein, 8 aa, Artificial Sequence
  LCDR3
KQSFNLFT

SEQ ID NO: 7 - protein, 121 aa, Artificial Sequence
  VH
QVQLVQSGAEVKKPGASVKVSCKASGYTFTDYWMHWVRQAPGQGLEWMGYINPSSGFTKYHQNFKDRVTMTRDTSISTAYMELSRLRSDDTAVYYCARQYDYDEDWYFDVWGQGTTVTVSS

SEQ ID NO: 8 - protein, 112 aa, Artificial Sequence
  VL
DIQMTQSPSSLSASVGDRVTITCKSSQSLLNSRTRKNFLAWYQQKPGKAPKLLIYWASTRESGVPSRFSGSGSGTDFTLTISSLQPEDFATYYCKQSFNLFTFGQGTKLEIK

SEQ ID NO: 9 - protein, 451 aa, Artificial Sequence
  HC
QVQLVQSGAEVKKPGASVKVSCKASGYTFTDYWMHWVRQAPGQGLEWMGYINPSSGFTKYHQNFKDRVTMTRDTSISTAYMELSRLRSDDTAVYYCARQYDYDEDWYFDVWGQGTTVTVSSASTKGPSVFPLAPSSKSTSGGTAALGCLVKDYFPEPVTVSWNSGALTSGVHTFPAVLQSSGLYSLSSVVTVPSSSLGTQTYICNVNHKPSNTKVDKKVEPKSCDKTHTCPPCPAPELLGGPSVFLFPPKPKDTLYITREPEVTCVVVDVSHEDPEVKFNWYVDGVEVHNAKTKPREEQYNSTYRVVSVLTVLHQDWLNGKEYKCKVSNKALPAPIEKTISKAKGQPREPQVYTLPPSRDELTKNQVSLTCLVKGFYPSDIAVEWESNGQPENNYKTTPPVLDSDGSFFLYSKLTVDKSRWQQGNVFSCSVMHEALHNHYTQKSLSLSPGK

SEQ ID NO: 10 - protein, 219 aa, Artificial Sequence
  LC
DIVMSQSPSSLSASVGDRVTITCKSSQSLLNSRTRKNFLAWYQQKPGKSPKLLIYWASTRESGVPDRFSGSGSGTDFTLTISSLQPEDFATYYCKQSFNLFTFGQGTKLEIKRTVAAPSVFIFPPSDEQLKSGTASVVCLLNNFYPREAKVQWKVDNALQSGNSQESVTEQDSKDSTYSLSSTLTLSKADYEKHKVYACEVTHQGLSSPVTKSFNRGEC